European Patent Application EP 4 198 124 A1, published June 21, 2023. Title: Engineered Cas9-Nucleases and Methods of Use Thereof. Applicant: The University of Hong Kong. Application US. The sequence listing filed with the application follows.

SEQUENCE LISTING (132 sequences)

SEQ ID NO: 1 - DNA, 26 bp, synthetic construct
  source 1..26: mol_type = other DNA
cacctacggcaatctgaccctgaagt

SEQ ID NO: 2 - DNA, 26 bp, synthetic construct
  source 1..26: mol_type = other DNA
cacctacggcaagctgaccctgaagt

SEQ ID NO: 3 - DNA, 26 bp, synthetic construct
  source 1..26: mol_type = other DNA
ggcgaggagctgttcaccggggtggt

SEQ ID NO: 4 - DNA, 20 bp, synthetic construct
  source 1..20: mol_type = other DNA
caactacggcaagctgaccc

SEQ ID NO: 5 - DNA, 20 bp, synthetic construct
  source 1..20: mol_type = other DNA
cacctacagcaagctgaccc

SEQ ID NO: 6 - DNA, 20 bp, synthetic construct
  source 1..20: mol_type = other DNA
cacctacggcaagctgaccc

SEQ ID NO: 7 - DNA, 20 bp, synthetic construct
  source 1..20: mol_type = other DNA
cacctacggcaagctgacct

SEQ ID NO: 8 - DNA, 20 bp, synthetic construct
  source 1..20: mol_type = other DNA
cacctacggcaagctgactc

SEQ ID NO: 9 - DNA, 20 bp, synthetic construct
  source 1..20: mol_type = other DNA
cacctacggcaagctgatcc

SEQ ID NO: 10 - DNA, 20 bp, synthetic construct
  source 1..20: mol_type = other DNA
cacctacggcaagctggccc

SEQ ID NO: 11 - DNA, 20 bp, synthetic construct
  source 1..20: mol_type = other DNA
cacctacggcaagctaaccc

SEQ ID NO: 12 - DNA, 20 bp, synthetic construct
  source 1..20: mol_type = other DNA
cacctacggcaagccgaccc

SEQ ID NO: 13 - DNA, 20 bp, synthetic construct
  source 1..20: mol_type = other DNA
cacctacggcaagttgaccc

SEQ ID NO: 14 - DNA, 20 bp, synthetic construct
  source 1..20: mol_type = other DNA
cacctacggcaaactgaccc

SEQ ID NO: 15 - DNA, 20 bp, synthetic construct
  source 1..20: mol_type = other DNA
cacctacggcaggctgaccc

SEQ ID NO: 16 - DNA, 20 bp, synthetic construct
  source 1..20: mol_type = other DNA
cacctacggcgagctgaccc

SEQ ID NO: 17 - DNA, 20 bp, synthetic construct
  source 1..20: mol_type = other DNA
cacctacggtaagctgaccc

SEQ ID NO: 18 - DNA, 20 bp, synthetic construct
  source 1..20: mol_type = other DNA
cacctacgacaagctgaccc

SEQ ID NO: 19 - DNA, 20 bp, synthetic construct
  source 1..20: mol_type = other DNA
cacctacagcaagctgaccc

SEQ ID NO: 20 - DNA, 20 bp, synthetic construct
  source 1..20: mol_type = other DNA
cacctatggcaagctgaccc

SEQ ID NO: 21 - DNA, 20 bp, synthetic construct
  source 1..20: mol_type = other DNA
cacctgcggcaagctgaccc

SEQ ID NO: 22 - DNA, 20 bp, synthetic construct
  source 1..20: mol_type = other DNA
cacccacggcaagctgaccc

SEQ ID NO: 23 - DNA, 20 bp, synthetic construct
  source 1..20: mol_type = other DNA
cacttacggcaagctgaccc

SEQ ID NO: 24 - DNA, 20 bp, synthetic construct
  source 1..20: mol_type = other DNA
catctacggcaagctgaccc

SEQ ID NO: 25 - DNA, 20 bp, synthetic construct
  source 1..20: mol_type = other DNA
cgcctacggcaagctgaccc

SEQ ID NO: 26 - DNA, 20 bp, synthetic construct
  source 1..20: mol_type = other DNA
tacctacggcaagctgaccc

SEQ ID NO: 27 - DNA, 20 bp, synthetic construct
  source 1..20: mol_type = other DNA
catttacggcaagctgaccc

SEQ ID NO: 28 - DNA, 20 bp, synthetic construct
  source 1..20: mol_type = other DNA
cgtctacggcaagctgaccc

SEQ ID NO: 29 - DNA, 20 bp, synthetic construct
  source 1..20: mol_type = other DNA
tgcctacggcaagctgaccc

SEQ ID NO: 30 - DNA, 21 bp, synthetic construct
  source 1..21: mol_type = other DNA
tggccaggctttggggaggcc

SEQ ID NO: 31 - DNA, 20 bp, synthetic construct
  source 1..20: mol_type = other DNA
gactaggaaggaggaggcct

SEQ ID NO: 32 - DNA, 20 bp, synthetic construct
  source 1..20: mol_type = other DNA
ggccaggctttggggaggcc

SEQ ID NO: 33 - DNA, 21 bp, synthetic construct
  source 1..21: mol_type = other DNA
gagagggacacacagatctat

SEQ ID NO: 34 - DNA, 21 bp, synthetic construct
  source 1..21: mol_type = other DNA
gttgccctaaggattaaatga

SEQ ID NO: 35 - DNA, 21 bp, synthetic construct
  source 1..21: mol_type = other DNA
gggtgagtgagtgtgtgcgtg

SEQ ID NO: 36 - DNA, 21 bp, synthetic construct
  source 1..21: mol_type = other DNA
gggtgagtgagtgtgtgcgta

SEQ ID NO: 37 - DNA, 21 bp, synthetic construct
  source 1..21: mol_type = other DNA
gggtgagtgagtgtgtgcgcg

SEQ ID NO: 38 - DNA, 21 bp, synthetic construct
  source 1..21: mol_type = other DNA
gggtgagtgagtgtgtgcatg

SEQ ID NO: 39 - DNA, 21 bp, synthetic construct
  source 1..21: mol_type = other DNA
gggtgagtgagtgtgtgtgtg

SEQ ID NO: 40 - DNA, 21 bp, synthetic construct
  source 1..21: mol_type = other DNA
gggtgagtgagtgtgtacgtg

SEQ ID NO: 41 - DNA, 21 bp, synthetic construct
  source 1..21: mol_type = other DNA
gggtgagtgagtgtgcgcgtg

SEQ ID NO: 42 - DNA, 21 bp, synthetic construct
  source 1..21: mol_type = other DNA
gggtgagtgagtgtatgcgtg

SEQ ID NO: 43 - DNA, 21 bp, synthetic construct
  source 1..21: mol_type = other DNA
gggtgagtgagtgcgtgcgtg

SEQ ID NO: 44 - DNA, 21 bp, synthetic construct
  source 1..21: mol_type = other DNA
gggtgagtgagtatgtgcgtg

SEQ ID NO: 45 - DNA, 21 bp, synthetic construct
  source 1..21: mol_type = other DNA
gggtgagtgagcgtgtgcgtg

SEQ ID NO: 46 - DNA, 21 bp, synthetic construct
  source 1..21: mol_type = other DNA
gggtgagtgaatgtgtgcgtg

SEQ ID NO: 47 - DNA, 21 bp, synthetic construct
  source 1..21: mol_type = other DNA
gggtgagtgggtgtgtgcgtg

SEQ ID NO: 48 - DNA, 21 bp, synthetic construct
  source 1..21: mol_type = other DNA
gggtgagtaagtgtgtgcgtg

SEQ ID NO: 49 - DNA, 21 bp, synthetic construct
  source 1..21: mol_type = other DNA
gggtgagcgagtgtgtgcgtg

SEQ ID NO: 50 - DNA, 21 bp, synthetic construct
  source 1..21: mol_type = other DNA
gggtgaatgagtgtgtgcgtg

SEQ ID NO: 51 - DNA, 21 bp, synthetic construct
  source 1..21: mol_type = other DNA
gggtgggtgagtgtgtgcgtg

SEQ ID NO: 52 - DNA, 21 bp, synthetic construct
  source 1..21: mol_type = other DNA
gggtaagtgagtgtgtgcgtg

SEQ ID NO: 53 - DNA, 21 bp, synthetic construct
  source 1..21: mol_type = other DNA
gggcgagtgagtgtgtgcgtg

SEQ ID NO: 54 - DNA, 21 bp, synthetic construct
  source 1..21: mol_type = other DNA
ggatgagtgagtgtgtgcgtg

SEQ ID NO: 55 - DNA, 21 bp, synthetic construct
  source 1..21: mol_type = other DNA
gagtgagtgagtgtgtgcgtg

SEQ ID NO: 56 - DNA, 21 bp, synthetic construct
  source 1..21: mol_type = other DNA
aggtgagtgagtgtgtgcgtg

SEQ ID NO: 57 - DNA, 21 bp, synthetic construct
  source 1..21: mol_type = other DNA
gcaaggcccggcgcacggtgg

SEQ ID NO: 58 - DNA, 21 bp, synthetic construct
  source 1..21: mol_type = other DNA
gcaaggcccggcgcacggtga

SEQ ID NO: 59 - DNA, 21 bp, synthetic construct
  source 1..21: mol_type = other DNA
gcaaggcccggcgcacggtag

SEQ ID NO: 60 - DNA, 21 bp, synthetic construct
  source 1..21: mol_type = other DNA
gcaaggcccggcgcacggcgg

SEQ ID NO: 61 - DNA, 21 bp, synthetic construct
  source 1..21: mol_type = other DNA
gcaaggcccggcgcacgatgg

SEQ ID NO: 62 - DNA, 21 bp, synthetic construct
  source 1..21: mol_type = other DNA
gcaaggcccggcgcacagtgg

SEQ ID NO: 63 - DNA, 21 bp, synthetic construct
  source 1..21: mol_type = other DNA
gcaaggcccggcgcatggtgg

SEQ ID NO: 64 - DNA, 21 bp, synthetic construct
  source 1..21: mol_type = other DNA
gcaaggcccggcgcgcggtgg

SEQ ID NO: 65 - DNA, 21 bp, synthetic construct
  source 1..21: mol_type = other DNA
gcaaggcccggcgtacggtgg

SEQ ID NO: 66 - DNA, 21 bp, synthetic construct
  source 1..21: mol_type = other DNA
gcaaggcccggcacacggtgg

SEQ ID NO: 67 - DNA, 21 bp, synthetic construct
  source 1..21: mol_type = other DNA
gcaaggcccggtgcacggtgg

SEQ ID NO: 68 - DNA, 21 bp, synthetic construct
  source 1..21: mol_type = other DNA
gcaaggcccgacgcacggtgg

SEQ ID NO: 69 - DNA, 21 bp, synthetic construct
  source 1..21: mol_type = other DNA
gcaaggcccagcgcacggtgg

SEQ ID NO: 70 - DNA, 21 bp, synthetic construct
  source 1..21: mol_type = other DNA
gcaaggcctggcgcacggtgg

SEQ ID NO: 71 - DNA, 21 bp, synthetic construct
  source 1..21: mol_type = other DNA
gcaaggctcggcgcacggtgg

SEQ ID NO: 72 - DNA, 21 bp, synthetic construct
  source 1..21: mol_type = other DNA
gcaaggtccggcgcacggtgg

SEQ ID NO: 73 - DNA, 21 bp, synthetic construct
  source 1..21: mol_type = other DNA
gcaagacccggcgcacggtgg

SEQ ID NO: 74 - DNA, 21 bp, synthetic construct
  source 1..21: mol_type = other DNA
gcaaagcccggcgcacggtgg

SEQ ID NO: 75 - DNA, 21 bp, synthetic construct
  source 1..21: mol_type = other DNA
gcagggcccggcgcacggtgg

SEQ ID NO: 76 - DNA, 21 bp, synthetic construct
  source 1..21: mol_type = other DNA
gcgaggcccggcgcacggtgg

SEQ ID NO: 77 - DNA, 21 bp, synthetic construct
  source 1..21: mol_type = other DNA
gtaaggcccggcgcacggtgg

SEQ ID NO: 78 - DNA, 21 bp, synthetic construct
  source 1..21: mol_type = other DNA
acaaggcccggcgcacggtgg

SEQ ID NO: 79 - protein, 1053 aa, Staphylococcus aureus
MKRNYILGLDIGITSVGYGIIDYETRDVIDAGVRLFKEANVENNEGRRSKRGARRLKRRRRHRIQRVKKLLFDYNLLTDHSELSGINPYEARVKGLSQKLSEEEFSAALLHLAKRRGVHNVNEVEEDTGNELSTKEQISRNSKALEEKYVAELQLERLKKDGEVRGSINRFKTSDYVKEAKQLLKVQKAYHQLDQSFIDTYIDLLETRRTYYEGPGEGSPFGWKDIKEWYEMLMGHCTYFPEELRSVKYAYNADLYNALNDLNNLVITRDENEKLEYYEKFQIIENVFKQKKKPTLKQIAKEILVNEEDIKGYRVTSTGKPEFTNLKVYHDIKDITARKEIIENAELLDQIAKILTIYQSSEDIQEELTNLNSELTQEEIEQISNLKGYTGTHNLSLKAINLILDELWHTNDNQIAIFNRLKLVPKKVDLSQQKEIPTTLVDDFILSPVVKRSFIQSIKVINAIIKKYGLPNDIIIELAREKNSKDAQKMINEMQKRNRQTNERIEEIIRTTGKENAKYLIEKIKLHDMQEGKCLYSLEAIPLEDLLNNPFNYEVDHIIPRSVSFDNSFNNKVLVKQEENSKKGNRTPFQYLSSSDSKISYETFKKHILNLAKGKGRISKTKKEYLLEERDINRFSVQKDFINRNLVDTRYATRGLMNLLRSYFRVNNLDVKVKSINGGFTSFLRRKWKFKKERNKGYKHHAEDALIIANADFIFKEWKKLDKAKKVMENQMFEEKQAESMPEIETEQEYKEIFITPHQIKHIKDFKDYKYSHRVDKKPNRELINDTLYSTRKDDKGNTLIVNNLNGLYDKDNDKLKKLINKSPEKLLMYHHDPQTYQKLKLIMEQYGDEKNPLYKYYEETGNYLTKYSKKDNGPVIKKIKYYGNKLNAHLDITDDYPNSRNKVVKLSLKPYRFDVYLDNGVYKFVTVKNLDVIKKENYYEVNSKCYEEAKKLKKISNQAEFIASFYNNDLIKINGELYRVIGVNNDLLNRIEVNMIDITYREYLENMNDKRPPRIIKTIASKTQSIKKYSTDILGNLYEVKSKKHPQIIKKG

SEQ ID NO: 80 - protein, 1053 aa, synthetic construct
MKRNYILGLDIGITSVGYGIIDYETRDVIDAGVRLFKEANVENNEGRRSKRGARRLKRRRRHRIQRVKKLLFDYNLLTDHSELSGINPYEARVKGLSQKLSEEEFSAALLHLAKRRGVHNVNEVEEDTGNELSTKEQISRNSKALEEKYVAELQLERLKKDGEVRGSINRFKTSDYVKEAKQLLKVQKAYHQLDQSFIDTYIDLLETRRTYYEGPGEGSPFGWKDIKEWYEMLMGHCTHFPEELRSVKYAYNADLYNALNDLNNLVITRDENEKLEYYEKFQIIENVFKQKKKPTLKQIAKEILVNEEDIKGYRVTSTGKPEFTNLKVYHDIKDITARKEIIENAELLDQIAKILTIYQSSEDIQEELTNLNSELTQEEIEQISNLKGYTGTHNLSLKAINLILDELWHTNDNQIAIFDRLKLVPKKVDLSQQKEIPTTLVDDFILSPVVKRSFIQSIKVINAIIKKYGLPNDIIIELAREKNSKDAQKMINEMQKRNAATNERIEEIIRTTGKENAKYLIEKIKLHDMQEGKCLYSLEAIPLEDLLNNPFNYEVDHIIPRSVSFDNSFNNKVLVKQEENSKKGNRTPFQYLSSSDSKISYETFKKHILNLAKGKGRISKTKKEYLLEERDINRFSVQKDFINRNLVDTRHATRGLMNLLRSYFRVNNLDVKVKSINGGFTSFLRRKWKFKKERNKGYKHHAEDALIIANADFIFKEWKKLDKAKKVMENQMFEEKQAESMPEIETEQEYKEIFITPHQIKHIKDFKDYKYSHRVDKKPNRKLINDTLYSTRKDDKGNTLIVNNLNGLYDKDNDKLKKLINKSPEKLLMYHHDPQTYQKLKLIMEQYGDEKNPLYKYYEETGNYLTKYSKKDNGPVIKKIKYYGNKLNAHLDITDDYPNSRNKVVKLSLKPYRFDVYLDNGVYKFVTVKNLDVIKKENYYEVNSKCYEEAKKLKKISNQAEFIASFYKNDLIKINGELYRVIGVNNDLLNRIEVNMIDITYREYLENMNDKRPPHIIKTIASKTQSIKKYSTDILGNLYEVKSKKHPQIIKKG

SEQ ID NO: 81 - protein, 1053 aa, synthetic construct
MKRNYILGLDIGITSVGYGIIDYETRDVIDAGVRLFKEANVENNEGRRSKRGARRLKRRRRHRIQRVKKLLFDYNLLTDHSELSGINPYEARVKGLSQKLSEEEFSAALLHLAKRRGVHNVNEVEEDTGNELSTKEQISRNSKALEEKYVAELQLERLKKDGEVRGSINRFKTSDYVKEAKQLLKVQKAYHQLDQSFIDTYIDLLETRRTYYEGPGEGSPFGWKDIKEWYEMLMGHCTHFPEELRSVKYAYNADLYNALNDLNNLVITRDENEKLEYYEKFQIIENVFKQKKKPTLKQIAKEILVNEEDIKGYRVTSTGKPEFTNLKVYHDIKDITARKEIIENAELLDQIAKILTIYQSSEDIQEELTNLNSELTQEEIEQISNLKGYTGTHNLSLKAINLILDELWHTNDNQIAIFDRLKLVPKKVDLSQQKEIPTTLVDDFILSPVVKRSFIQSIKVINAIIKKYGLPNDIIIELAREKNSKDAQKMINEMQKRNRQTNERIEEIIRTTGKENAKYLIEKIKLHDMQEGKCLYSLEAIPLEDLLNNPFNYEVDHIIPRSVSFDNSFNNKVLVKQEENSKKGNRTPFQYLSSSDSKISYETFKKHILNLAKGKGRISKTKKEYLLEERDINRFSVQKDFINRNLVDTRYATAALMNLLRSYFRVNNLDVKVKSINGGFTSFLRRKWKFKKERNKGYKHHAEDALIIANADFIFKEWKKLDKAKKVMENQMFEEKQAESMPEIETEQEYKEIFITPHQIKHIKDFKDYKYSHRVDKKPNRKLINDTLYSTRKDDKGNTLIVNNLNGLYDKDNDKLKKLINKSPEKLLMYHHDPQTYQKLKLIMEQYGDEKNPLYKYYEETGNYLTKYSKKDNGPVIKKIKYYGNKLNAHLDITDDYPNSRNKVVKLSLKPYRFDVYLDNGVYKFVTVKNLDVIKKENYYEVNSKCYEEAKKLKKISNQAEFIASFYKNDLIKINGELYRVIGVNNDLLNRIEVNMIDITYREYLENMNDKRPPHIIKTIASKTQSIKKYSTDILGNLYEVKSKKHPQIIKKG

SEQ ID NO: 82 - DNA, 22 bp, synthetic construct
  source 1..22: mol_type = other DNA
gtgtggttccagaaccggagga

SEQ ID NO: 83 - DNA, 21 bp, synthetic construct
  source 1..21: mol_type = other DNA
gctcagcctgagtgttgaggc

SEQ ID NO: 84 - protein, 18 aa, synthetic construct
TYRNTNNQNRQGYRGKKH

SEQ ID NO: 85 - protein, 18 aa, synthetic construct
AHRNATNQGRQGYAAKKH

SEQ ID NO: 86 - protein, 18 aa, synthetic construct
THRNTTNQSAAGYAAKKH

SEQ ID NO: 87 - protein, 18 aa, synthetic construct
THRNTNNRDRQGHRGKKH

SEQ ID NO: 88 - protein, 18 aa, synthetic construct
THRNTTNQDRQGYAAKKH

SEQ ID NO: 89 - protein, 18 aa, synthetic construct
THRNTANRDRQGYAAKKH

SEQ ID NO: 90 - protein, 18 aa, synthetic construct
THRNTNNQDAAGHRGKKH

SEQ ID NO: 91 - protein, 18 aa, synthetic construct
THRNTNNQDRQGYAAKKH

SEQ ID NO: 92 - protein, 18 aa, synthetic construct
TYANTNNQDRQGYAAKKH

SEQ ID NO: 93 - protein, 18 aa, synthetic construct
TYRNTNNQDRQGYAAKKH

SEQ ID NO: 94 - protein, 18 aa, synthetic construct
THANTNNQDRQGYAAKKH

SEQ ID NO: 95 - protein, 18 aa, synthetic construct
THRNTNAQARQGYAGKKH

SEQ ID NO: 96 - protein, 18 aa, synthetic construct
TYANTNAQARQGYAGKKH

SEQ ID NO: 97 - protein, 18 aa, synthetic construct
TYRNTNAQARQGYAGKKH

SEQ ID NO: 98 - protein, 18 aa, synthetic construct
THANTNAQARQGYAGKKH

SEQ ID NO: 99 - protein, 18 aa, synthetic construct
TYARNTAQARQGYAGENR

SEQ ID NO: 100 - protein, 18 aa, synthetic construct
TYRNTNNQNRQGYRGENR

SEQ ID NO: 101 - DNA, 21 bp, synthetic construct
  source 1..21: mol_type = other DNA
gcaaccacaaacccacgaggg

SEQ ID NO: 102 - DNA, 21 bp, synthetic construct
  source 1..21: mol_type = other DNA
ggctctccgaggagaaggcca

SEQ ID NO: 103 - DNA, 21 bp, synthetic construct
  source 1..21: mol_type = other DNA
aaacgacccccaaagaaccgt

SEQ ID NO: 104 - DNA, 21 bp, synthetic construct
  source 1..21: mol_type = other DNA
agtctgaaagagccaaatcgg

SEQ ID NO: 105 - DNA, 21 bp, synthetic construct
  source 1..21: mol_type = other DNA
gtatgcaggcatcctcagcta

SEQ ID NO: 106 - DNA, 21 bp, synthetic construct
  source 1..21: mol_type = other DNA
gcctgcggacatcgtcgggca

SEQ ID NO: 107 - DNA, 21 bp, synthetic construct
  source 1..21: mol_type = other DNA
gcctgcggatatcgtcgggca

SEQ ID NO: 108 - DNA, 21 bp, synthetic construct
  source 1..21: mol_type = other DNA
gcccgcggacatcgtcgggca

SEQ ID NO: 109 - DNA, 21 bp, synthetic construct
  source 1..21: mol_type = other DNA
cgtcgggcgctcacaccgtgc

SEQ ID NO: 110 - DNA, 21 bp, synthetic construct
  source 1..21: mol_type = other DNA
cgtcgggcgttcacaccgtgc

SEQ ID NO: 111 - DNA, 38 bp, synthetic construct
  source 1..38: mol_type = other DNA
gntnttaattgagttgtcatatgttaataacggtnant

SEQ ID NO: 112 - DNA, 38 bp, synthetic construct
  source 1..38: mol_type = other DNA
antnaccgttattaacatatgacaactcaattaananc

SEQ ID NO: 113 - DNA, 20 bp, synthetic construct
  source 1..20: mol_type = other DNA
ggagcagctggtcagagggg

SEQ ID NO: 114 - DNA, 22 bp, synthetic construct
  source 1..22: mol_type = other DNA
ccatagggaagggggacactgg

SEQ ID NO: 115 - DNA, 20 bp, synthetic construct
  source 1..20: mol_type = other DNA
tccagatggcacattgtcag

SEQ ID NO: 116 - DNA, 20 bp, synthetic construct
  source 1..20: mol_type = other DNA
agggagcaggaaagtgaggt

SEQ ID NO: 117 - DNA, 20 bp, synthetic construct
  source 1..20: mol_type = other DNA
gggccgggaaagagttgctg

SEQ ID NO: 118 - DNA, 22 bp, synthetic construct
  source 1..22: mol_type = other DNA
gccctacatctgctctccctcc

SEQ ID NO: 119 - DNA, 20 bp, synthetic construct
  source 1..20: mol_type = other DNA
gactcaaacccagaagccca

SEQ ID NO: 120 - DNA, 20 bp, synthetic construct
  source 1..20: mol_type = other DNA
agccacctctccatcctctt

SEQ ID NO: 121 - DNA, 20 bp, synthetic construct
  source 1..20: mol_type = other DNA
ccggccatttcactctgact

SEQ ID NO: 122 - DNA, 20 bp, synthetic construct
  source 1..20: mol_type = other DNA
ttgctgctagcttccctgtc

SEQ ID NO: 123 - DNA, 22 bp, synthetic construct
  source 1..22: mol_type = other DNA
gaggtgtccacttacacaggaa

SEQ ID NO: 124 - DNA, 20 bp, synthetic construct
  source 1..20: mol_type = other DNA
tcaaaatcgcccctgtgagg

SEQ ID NO: 125 - DNA, 20 bp, synthetic construct
  source 1..20: mol_type = other DNA
acagacagcgtttggttgac

SEQ ID NO: 126 - DNA, 22 bp, synthetic construct
  source 1..22: mol_type = other DNA
gagccctagacagggtttttat

SEQ ID NO: 127 - DNA, 20 bp, synthetic construct
  source 1..20: mol_type = other DNA
tcactggcgttactgactgc

SEQ ID NO: 128 - DNA, 20 bp, synthetic construct
  source 1..20: mol_type = other DNA
tgtgttggagctcatggacg

SEQ ID NO: 129 - DNA, 20 bp, synthetic construct
  source 1..20: mol_type = other DNA
cacctacggcaagctgaccc

SEQ ID NO: 130 - DNA, 20 bp, synthetic construct
  source 1..20: mol_type = other DNA
cacctacggcaatctgaccc

SEQ ID NO: 131 - DNA, 3156 bp, synthetic construct
  source 1..3156: mol_type = other DNA
aagcggaactacatcctgggcctggacatcggcatcaccagcgtgggctacggcatcatcgactacgagacacgggacgtgatcgatgccggcgtgcggctgttcaaagaggccaacgtggaaaacaacgagggcaggcggagcaagagaggcgccagaaggctgaagcggcggaggcggcatagaatccagagagtgaagaagctgctgttcgactacaacctgctgaccgaccacagcgagctgagcggcatcaacccctacgaggccagagtgaagggcctgagccagaagctgagcgaggaagagttctctgccgccctgctgcacctggccaagagaagaggcgtgcacaacgtgaacgaggtggaagaggacaccggcaacgagctgtccaccaaagagcagatcagccggaacagcaaggccctggaagagaaatacgtggccgaactgcagctggaacggctgaagaaagacggcgaagtgcggggcagcatcaacagattcaagaccagcgactacgtgaaagaagccaaacagctgctgaaggtgcagaaggcctaccaccagctggaccagagcttcatcgacacctacatcgacctgctggaaacccggcggacctactatgagggacctggcgagggcagccccttcggctggaaggacatcaaagaatggtacgagatgctgatgggccactgcacccacttccccgaggaactgcggagcgtgaagtacgcctacaacgccgacctgtacaacgccctgaacgacctgaacaatctcgtgatcaccagggacgagaacgagaagctggaatattacgagaagttccagatcatcgagaacgtgttcaagcagaagaagaagcccaccctgaagcagatcgccaaagaaatcctcgtgaacgaagaggatattaagggctacagagtgaccagcaccggcaagcccgagttcaccaacctgaaggtgtaccacgacatcaaggacattaccgcccggaaagagattattgagaacgccgagctgctggatcagattgccaagatcctgaccatctaccagagcagcgaggacatccaggaagaactgaccaatctgaactccgagctgacccaggaagagatcgagcagatctctaatctgaagggctataccggcacccacaacctgagcctgaaggccatcaacctgatcctggacgagctgtggcacaccaacgacaaccagatcgctatcttcgaccggctgaagctggtgcccaagaaggtggacctgtcccagcagaaagagatccccaccaccctggtggacgacttcatcctgagccccgtcgtgaagagaagcttcatccagagcatcaaagtgatcaacgccatcatcaagaagtacggcctgcccaacgacatcattatcgagctggcccgcgagaagaactccaaggacgcccagaaaatgatcaacgagatgcagaagcggaacgccgccaccaacgagcggatcgaggaaatcatccggaccaccggcaaagagaacgccaagtacctgatcgagaagatcaagctgcacgacatgcaggaaggcaagtgcctatacagcctggaagccatccctctggaagatctgctgaacaaccccttcaactatgaggtggaccacatcatccccagaagcgtgtccttcgacaacagcttcaacaacaaggtgctcgtgaagcaggaagaaaacagcaagaagggcaaccggaccccattccagtacctgagcagcagcgacagcaagatcagctacgaaaccttcaagaagcacatcctgaatctggccaagggcaagggcagaatcagcaagaccaagaaagagtatctgctggaagaacgggacatcaacaggttctccgtgcagaaagacttcatcaaccggaacctggtggataccagacacgccaccagaggcctgatgaacctgctgcggagctacttcagagtgaacaacctggacgtgaaagtgaagtccatcaatggcggcttcaccagctttctgcggcggaagtggaagtttaagaaagagcggaacaaggggtacaagcaccacgccgaggacgccctgatcattgccaacgccgatttcatcttcaaagagtggaagaaactggacaaggccaaaaaagtgatggaaaaccagatgttcgaggaaaagcaggccgagagcatgcccgagatcgaaaccgagcaggagtacaaagagatcttcatcaccccccaccagatcaagcacattaaggacttcaaggactacaagtacagccatcgggtggacaagaagcctaatagaaagctgattaacgacaccctgtactccacccggaaggacgacaagggcaacaccctgatcgtgaacaatctgaacggcctgtacgacaaggacaatgacaagctgaaaaagctgatcaacaagagccccgaaaagctgctgatgtaccaccacgacccccagacctaccagaaactgaagctgattatggaacagtacggcgacgagaagaatcccctgtacaagtactacgaggaaaccgggaactacctgaccaagtactccaaaaaggacaacggccccgtgatcaagaagattaagtattacggcaacaaactgaacgcccatctggacatcaccgacgactaccccaacagcagaaacaaggtcgtgaagctgtccctgaagccctacagattcgacgtgtacctggacaatggcgtgtacaagttcgtgaccgtgaagaatctggatgtgatcaaaaaagaaaactactacgaagtgaatagcaagtgctatgaggaagctaagaagctgaagaagatcagcaaccaggccgagtttatcgcctccttctacaagaacgatctgatcaagatcaacggcgagctgtatagagtgatcggcgtgaacaacgacctgctgaaccggatcgaagtgaacatgatcgacatcacctaccgcgagtacctggaaaacatgaacgacaagaggcccccccacatcattaagacaatcgcctccaagacccagagcattaagaagtacagcacagacattctgggcaacctgtatgaagtgaaatctaagaagcaccctcagatcatcaaaaagggc

SEQ ID NO: 132 - DNA, 3156 bp, synthetic construct
  source 1..3156: mol_type = other DNA
aagcggaactacatcctgggcctggacatcggcatcaccagcgtgggctacggcatcatcgactacgagacacgggacgtgatcgatgccggcgtgcggctgttcaaagaggccaacgtggaaaacaacgagggcaggcggagcaagagaggcgccagaaggctgaagcggcggaggcggcatagaatccagagagtgaagaagctgctgttcgactacaacctgctgaccgaccacagcgagctgagcggcatcaacccctacgaggccagagtgaagggcctgagccagaagctgagcgaggaagagttctctgccgccctgctgcacctggccaagagaagaggcgtgcacaacgtgaacgaggtggaagaggacaccggcaacgagctgtccaccaaagagcagatcagccggaacagcaaggccctggaagagaaatacgtggccgaactgcagctggaacggctgaagaaagacggcgaagtgcggggcagcatcaacagattcaagaccagcgactacgtgaaagaagccaaacagctgctgaaggtgcagaaggcctaccaccagctggaccagagcttcatcgacacctacatcgacctgctggaaacccggcggacctactatgagggacctggcgagggcagccccttcggctggaaggacatcaaagaatggtacgagatgctgatgggccactgcacccacttccccgaggaactgcggagcgtgaagtacgcctacaacgccgacctgtacaacgccctgaacgacctgaacaatctcgtgatcaccagggacgagaacgagaagctggaatattacgagaagttccagatcatcgagaacgtgttcaagcagaagaagaagcccaccctgaagcagatcgccaaagaaatcctcgtgaacgaagaggatattaagggctacagagtgaccagcaccggcaagcccgagttcaccaacctgaaggtgtaccacgacatcaaggacattaccgcccggaaagagattattgagaacgccgagctgctggatcagattgccaagatcctgaccatctaccagagcagcgaggacatccaggaagaactgaccaatctgaactccgagctgacccaggaagagatcgagcagatctctaatctgaagggctataccggcacccacaacctgagcctgaaggccatcaacctgatcctggacgagctgtggcacaccaacgacaaccagatcgctatcttcgaccggctgaagctggtgcccaagaaggtggacctgtcccagcagaaagagatccccaccaccctggtggacgacttcatcctgagccccgtcgtgaagagaagcttcatccagagcatcaaagtgatcaacgccatcatcaagaagtacggcctgcccaacgacatcattatcgagctggcccgcgagaagaactccaaggacgcccagaaaatgatcaacgagatgcagaagcggaaccggcagaccaacgagcggatcgaggaaatcatccggaccaccggcaaagagaacgccaagtacctgatcgagaagatcaagctgcacgacatgcaggaaggcaagtgcctatacagcctggaagccatccctctggaagatctgctgaacaaccccttcaactatgaggtggaccacatcatccccagaagcgtgtccttcgacaacagcttcaacaacaaggtgctcgtgaagcaggaagaaaacagcaagaagggcaaccggaccccattccagtacctgagcagcagcgacagcaagatcagctacgaaaccttcaagaagcacatcctgaatctggccaagggcaagggcagaatcagcaagaccaagaaagagtatctgctggaagaacgggacatcaacaggttctccgtgcagaaagacttcatcaaccggaacctggtggataccagatacgccaccgccgccctgatgaacctgctgcggagctacttcagagtgaacaacctggacgtgaaagtgaagtccatcaatggcggcttcaccagctttctgcggcggaagtggaagtttaagaaagagcggaacaaggggtacaagcaccacgccgaggacgccctgatcattgccaacgccgatttcatcttcaaagagtggaagaaactggacaaggccaaaaaagtgatggaaaaccagatgttcgaggaaaagcaggccgagagcatgcccgagatcgaaaccgagcaggagtacaaagagatcttcatcaccccccaccagatcaagcacattaaggacttcaaggactacaagtacagccatcgggtggacaagaagcctaatagaaagctgattaacgacaccctgtactccacccggaaggacgacaagggcaacaccctgatcgtgaacaatctgaacggcctgtacgacaaggacaatgacaagctgaaaaagctgatcaacaagagccccgaaaagctgctgatgtaccaccacgacccccagacctaccagaaactgaagctgattatggaacagtacggcgacgagaagaatcccctgtacaagtactacgaggaaaccgggaactacctgaccaagtactccaaaaaggacaacggccccgtgatcaagaagattaagtattacggcaacaaactgaacgcccatctggacatcaccgacgactaccccaacagcagaaacaaggtcgtgaagctgtccctgaagccctacagattcgacgtgtacctggacaatggcgtgtacaagttcgtgaccgtgaagaatctggatgtgatcaaaaaagaaaactactacgaagtgaatagcaagtgctatgaggaagctaagaagctgaagaagatcagcaaccaggccgagtttatcgcctccttctacaagaacgatctgatcaagatcaacggcgagctgtatagagtgatcggcgtgaacaacgacctgctgaaccggatcgaagtgaacatgatcgacatcacctaccgcgagtacctggaaaacatgaacgacaagaggcccccccacatcattaagacaatcgcctccaagacccagagcattaagaagtacagcacagacattctgggcaacctgtatgaagtgaaatctaagaagcaccctcagatcatcaaaaagggc